European Patent Application EP 4 375 365 A1, published May 29, 2024. Title: Novel Lactobacillus paracasei ATG-E1 strain, and composition comprising thereof for preventing or treating respiratory disease. Applicant: AtoGen Co., Ltd. The sequence listing filed with the application follows.

SEQUENCE LISTING (1 sequence)

SEQ ID NO: 1 - DNA, 1435 bp, Lactobacillus paracasei
agtcgaacgagttctcgttgatgatcggtgcttgcaccgagattcaacatggaacgagtggcggacgggtgagtaacacgtgggtaacctgcccttaagtgggggataacatttggaaacagatgctaataccgcatagatccaagaaccgcatggttcttggctgaaagatggcgtaagctatcgcttttggatggacccgcggcgtattagagttggtgaggtaatggctcaccaaggcgatgatacgtagccgaactgagaggttgatcggccacattgggactgagacacggcccaaactcctacgggaggcagcagtagggaatcttccacaatggacgcaagtctgatggagcaacgccgcgtgagtgaagaaggctttcgggtcgtaaaactctgttgttggagaagaatggtcggcaagtaactgttgtcggcgtgacggtatccaaccagaaagccacggctaactacgtgccagcagccgcggtaatacgtaggtggcaagcgttatccggatttattgggcgtaaagcgagcgcaggcggttttttaagtctgatgtgaaagccctcggcttaaccgaggaagcgcatcggaaactgggaaacttgagtgcagaagaggacagtggaactccatgtgtagcggtgaaatgcgtagatatatggaagaacaccagtggcgaaggcggctgtctggtctgtaactgacgctgaggctcgaaagcatgggtagcgaacaggattagataccctggtagtccatgccgtaaacgatgaatgctaggtgttggagggtttccgcccttcagtgccgcagctaacgcattaagcattccgcctggggagtacgaccgcaaggttgaaactcaaaggaattgacgggggcccgcacaagcggtggagcatgtggtttaattcgaagcaacgcgaagaaccttaccaggtcttgacatcttttgatcacctgagagatcaggtttccccttcgggggcaaaatgacaggtggtgcatggttgtcgtcagctcgtgtcgtgagatgttgggttaagtcccgcaacgagcgcaacccttatgactagttgccagcatttagttgggcactctagtaagactgccggtgacaaaccggaggaaggtggggatgacgtcaaatcatcatgccccttatgacctgggctacacacgtgctacaatggatggtacaacgagttgcgagaccgcgaggtcaagctaatctcttaaagccattctcagttcggactgtaggctgcaactcgcctacacgaagtcggaatcgctagtaatcgcggatcagcacgccgcggtgaatacgttcccgggccttgtacacaccgcccgtcacaccatgagagtttgtaacacccgaagccggtggcgtaacccttttagggagcgagccgtctaa